European Patent Application EP 4 372 095 A1, published May 22, 2024. Title: Method for producing plasmid DNA using Escherichia coli. Applicant: Kaneka Corporation Kaneka Eurogentec S. A. Universite catholique de Louvain. The sequence listing filed with the application follows.

SEQUENCE LISTING (83 sequences)

SEQ ID NO: 1 - DNA, 459 bp, Escherichia coli
tgttcttccaacaagaacgccagcaatgacggcagcgaaggcatgctgggtgccggcactggtatggatgcgaacggcggcaacggcaacatgtcttccgaagagcaggctcgtctgcaaatgcaacagctgcagcagaacaacatcgtttacttcgatctggacaagtacgatatccgttctgacttcgctcaaatgctggatgcacatgcaaacttcctgcgtagcaacccgtcttacaaagtcaccgtagaaggtcacgcggacgaacgtggtactccggaatacaacatctccctgggtgaacgtcgtgcgaacgccgttaagatgtacctgcagggtaaaggcgtttctgcagaccagatctccatcgtttcttacggtaaagaaaaacctgcagtactgggtcatgacgaagcggcatactccaaaaaccgtcgtgcggtactggtttactaa

SEQ ID NO: 2 - DNA, 63 bp, Escherichia coli
atgcaactgaacaaagtgctgaaagggctgatgattgctctgcctgttatggcaattgcggca

SEQ ID NO: 3 - DNA, 177 bp, Escherichia coli
tgctccagcaacgctaaaatcgatcagctgtcttctgacgttcagactctgaacgctaaagttgaccagctgagcaacgacgtgaacgcaatgcgttccgacgttcaggctgctaaagatgacgcagctcgtgctaaccagcgtctggacaacatggctactaaataccgcaagtaa

SEQ ID NO: 4 - DNA, 60 bp, Escherichia coli
atgaaagctactaaactggtactgggcgcggtaatcctgggttctactctgctggcaggt

SEQ ID NO: 5 - DNA, 978 bp, Escherichia coli
gctccgaaagataacacctggtacactggtgctaaactgggctggtcccagtaccatgacactggtttcatcaacaacaatggcccgacccatgaaaaccaactgggcgctggtgcttttggtggttaccaggttaacccgtatgttggctttgaaatgggttacgactggttaggtcgtatgccgtacaaaggcagcgttgaaaacggtgcatacaaagctcagggcgttcaactgaccgctaaactgggttacccaatcactgacgacctggacatctacactcgtctgggtggcatggtatggcgtgcagacactaaatccaacgtttatggtaaaaaccacgacaccggcgtttctccggtcttcgctggcggtgttgagtacgcgatcactcctgaaatcgctacccgtctggaataccagtggaccaacaacatcggtgacgcacacaccatcggcactcgtccggacaacggcatgctgagcctgggtgtttcctaccgtttcggtcagggcgaagcagctccagtagttgctccggctccagctccggcaccggaagtacagaccaagcacttcactctgaagtctgacgttctgttcaacttcaacaaagcaaccctgaaaccggaaggtcaggctgctctggatcagctgtacagccagctgagcaacctggatccgaaagacggttccgtagttgttctgggttacaccgaccgcatcggttctgacgcttacaaccagggtctgtccgagcgccgtgctcagtctgttgttgattacctgatctccaaaggtatcccggcagacaagatctccgcacgtggtatgggcgaatccaacccggttactggcaacacctgtgacaacgtgaaacagcgtgctgcactgatcgactgcctggctccggatcgtcgcgtagagatcgaagttaaaggtatcaaagacgttgtaactcagccgcaggcttaa

SEQ ID NO: 6 - DNA, 63 bp, Escherichia coli
atgaaaaagacagctatcgcgattgcagtggcactggctggtttcgctaccgtagcgcaggcc

SEQ ID NO: 7 - DNA, 1266 bp, Escherichia coli
gtgtcaaaggcaaccgaacaaaacgacaagctcaagcgggcgataattatttcagcagtgctgcatgtcatcttatttgcggcgctgatctggagttcgttcgatgagaatatagaagcttcagccggaggcggcggtggttcgtccatcgacgctgtcatggttgattcaggtgcggtagttgagcagtacaaacgcatgcaaagccaggaatcaagcgcgaagcgttctgatgaacagcgcaagatgaaggaacagcaggctgctgaagaactgcgtgagaaacaagcggctgaacaggaacgcctgaagcaacttgagaaagagcggttagcggctcaggagcagaaaaagcaggctgaagaagccgcaaaacaggccgagttaaagcagaagcaagctgaagaggcggcagcgaaagcggcggcagatgctaaagcgaaggccgaagcagatgctaaagctgcggaagaagcagcgaagaaagcggctgcagacgcaaagaaaaaagcagaagcagaagccgccaaagccgcagccgaagcgcagaaaaaagccgaggcagccgctgcggcactgaagaagaaagcggaagcggcagaagcagctgcagctgaagcaagaaagaaagcggcaactgaagctgctgaaaaagccaaagcagaagctgagaagaaagcggctgctgaaaaggctgcagctgataagaaagcggcagcagagaaagctgcagccgacaaaaaagcagcagaaaaagcggctgctgaaaaggcagcagctgataagaaagcagcggcagaaaaagccgccgcagacaaaaaagcggcagcggcaaaagctgcagctgaaaaagccgctgcagcaaaagcggccgcagaggcagatgatattttcggtgagctaagctctggtaagaatgcaccgaaaacggggggaggggcgaaagggaacaatgcttcgcctgccgggagtggtaatactaaaaacaatggcgcatcaggggccgatatcaataactatgccgggcagattaaatctgctatcgaaagtaagttctatgacgcatcgtcctatgcaggcaaaacctgtacgctgcgcataaaactggcacccgatggtatgttactggatatcaaacctgaaggtggcgatcccgcactttgtcaggctgcgttggcagcagctaaacttgcgaagatcccgaaaccaccaagccaggcagtatatgaagtgttcaaaaacgcgccattggacttcaaaccgtaa

SEQ ID NO: 8 - DNA, 1230 bp, Escherichia coli
gaagtccgcattgtgatcgacagcggtgtagattccggtcgtcctattggtgttgttcctttccagtgggcggggcctggtgcggcacctgaagatattggcggcatcgttgctgctgacttgcgtaacagcggtaaatttaatccgttagatcgcgctcgtctgccacagcagccgggtagtgcgcaggaagtacaaccagctgcatggtccgcactgggcattgacgctgtagttgtcggtcaggtcactccgaatccggatggttcttacaatgttgcttatcaacttgttgacactggcggcgcaccgggtactgtacttgctcagaactcgtacaaagtgaacaagcagtggctgcgttatgctggtcataccgccagtgatgaagtgtttgaaaaactgaccggcattaaaggtgcgttccgtactcgtattgcctacgttgttcagaccaacggcggtcagttcccgtatgaactgcgcgtatctgactatgacggttacaaccagtttgtcgttcaccgttcaccgcagccgctgatgtctccggcgtggtcaccagacggttctaaactggcttatgtgaccttcgaaagcggtcgttccgcgctggttattcagacgctggcaaatggcgctgtacgtcaggtggcttcattcccgcgtcacaacggtgcacctgcattctcgccagacggcagcaaactggcattcgccttgtcgaaaaccggtagtctgaacctgtacgtaatggatttggcttctggtcagatccgccaggtgactgatggtcgcagtaacaataccgaaccgacctggttcccggatagccagaacctggcatttacttctgaccaggccggtcgtccgcaggtttataaagtgaatatcaacggcggtgcgccacaacgtattacctgggaaggttcgcagaaccaggatgcggatgtcagcagcgacggtaaatttatggtaatggtcagctccaatggtgggcagcagcacattgccaaacaagatctggcaacgggaggcgtacaagttctgtcgtccacgttcctggatgaaacgccaagtctggcacctaacggcactatggtaatctacagctcttctcaggggatgggatccgtgctgaatttggtttctacagatgggcgtttcaaagcgcgtcttccggcaactgatggacaggtcaaattccctgcctggtcgccgtatctgtga

SEQ ID NO: 9 - DNA, 63 bp, Escherichia coli
atgaagcaggcattacgagtagcatttggttttctcatactgtgggcatcagttctgcatgct

SEQ ID NO: 10 - DNA, 489 bp, Escherichia coli
tgtagtgcaaataacaccgcaaagaatatgcatcctgagacacgtgcagtgggtagtgaaacatcatcactgcaagcttctcaggatgaatttgaaaacctggttcgtaatgtcgacgtaaaatcgcgaattatggatcagtatgctgactggaaaggcgtacgttatcgtctgggcggcagcactaaaaaaggtatcgattgttctggtttcgtacagcgtacattccgtgagcaatttggcttagaacttccgcgttcgacttacgaacagcaggaaatgggtaaatctgtttcccgcagtaatttgcgtacgggtgatttagttctgttccgtgccggttcaacgggacgccatgtcggtatttatatcggcaacaatcagtttgtccatgcttccaccagcagtggtgttattatttccagcatgaatgaaccgtactggaagaagcgttacaacgaagcacgccgggttctcagccgcagctaa

SEQ ID NO: 11 - DNA, 78 bp, Escherichia coli
atggtcaaatctcaaccgattttgagatatatcttgcgcgggattcccgcgattgcagtagcggttctgctttctgca

SEQ ID NO: 12 - DNA, 831 bp, Escherichia coli
tgcagtaatacttcctggcgtaaaagtgaagtcctcgcggtaccattgcaaccgactttacagcaggaagtgattctggcacgtatggaacaaatccttgccagtcgggctttaaccgatgacgaacgcgcacagcttttatatgagcgcggagtgttgtatgatagtctcggtctgagggcattagcgcgtaacgatttttcgcaagcgctggcaatccgaccggatatgcctgaagtattcaattacttaggcatatatttaacgcaggcaggcaattttgatgctgcctatgaagcgtttgattctgtacttgagcttgatccaacttacaactacgcgcacttgaatcgcgggatcgcattatattacggcggtcgtgacaagttagcgcaagatgatctgctggcgttttatcaagacgatcccaatgatcctttccgtagtctgtggctttatctcgccgagcagaagctcgatgagaagcaggctaaagaagtgttgaaacagcacttcgaaaaatcggataaggaacagtggggatggaacattgtcgagttctacctgggcaacattagcgaacaaacgttaatggaaaggctcaaggcggacgcaacggataacacctcgctcgctgagcatctcagtgaaaccaacttctatttaggtaagtactacctaagtctgggggatttggacagcgccacggcactgttcaaactggcggttgccaacaacgttcataactttgttgagcaccgatacgcattgttggaattatcgctcctgggccaggaccaagatgacctggcagaatcggaccagcaatag

SEQ ID NO: 13 - DNA, 54 bp, Escherichia coli
atgaagccttttttgcgctggtgtttcgttgcgacagcacttacgcttgcagga

SEQ ID NO: 14 - DNA, 717 bp, Escherichia coli
atgcagaccccgcacattcttatcgttgaagacgagttggtaacacgcaacacgttgaaaagtattttcgaagcggaaggctatgatgttttcgaagcgacagatggcgcggaaatgcatcagatcctctctgaatatgacatcaacctggtgatcatggatatcaatctgccgggtaagaacggtcttctgttagcgcgtgaactgcgcgagcaggcgaatgttgcgttgatgttcctgactggccgtgacaacgaagtcgataaaattctcggcctcgaaatcggtgcagatgactacatcaccaaaccgttcaacccgcgtgaactgacgattcgtgcacgcaacctactgtcccgtaccatgaatctgggtactgtcagcgaagaacgtcgtagcgttgaaagctacaagttcaatggttgggaactggacatcaacagccgttcgttgatcggccctgatggcgagcagtacaagctgccgcgcagcgagttccgcgccatgcttcacttctgtgaaaacccaggcaaaattcagtcccgtgctgaactgctgaagaaaatgaccggccgtgagctgaaaccgcacgaccgtactgtagacgtgacgatccgccgtattcgtaaacatttcgaatctacgccggatacgccggaaatcatcgccaccattcacggtgaaggttatcgcttctgcggtgatctggaagattaa

SEQ ID NO: 15 - DNA, 681 bp, Escherichia coli
tgctcggggtcaaaggaagaagtacctgataatccgccaaatgaaatttacgcgactgcacaacaaaagctgcaggacggtaactggagacaggcaataacgcaactggaagcgttagataatcgctatccgtttggtccgtattcgcagcaggtgcagctggatctcatctacgcctactataaaaacgccgatttgccgttagcacaggctgccatcgatcgttttattcgccttaacccgacccatccgaatatcgattatgtcatgtacatgcgtggcctgaccaatatggcgctggatgacagtgcgctgcaagggttctttggcgtcgatcgtagcgatcgcgatcctcaacatgcacgagctgcgtttagtgacttttccaaactggtgcgcggctatccgaacagtcagtacaccaccgatgccaccaaacgtctggtattcctgaaagatcgtctggcgaaatatgaatactccgtggccgagtactatacagaacgtggcgcatgggttgccgtcgttaaccgcgtagaaggcatgttgcgcgactacccggatacccaggctacgcgtgatgcgctgccgctgatggaaaatgcataccgtcagatgcagatgaatgcgcaagctgaaaaagtagcgaaaatcatcgccgcaaacagcagcaatacataa

SEQ ID NO: 16 - DNA, 57 bp, Escherichia coli
atgacgcgcatgaaatatctggtggcagccgccacactaagcctgtttttggcgggt

SEQ ID NO: 17 - DNA, 876 bp, Escherichia coli
tgtaattctgcgctgttagatcccaaaggacagattggtctggagcaacgttcactgatactgacggcatttggcctgatgttgattgtcgttattcccgcaatcttgatggctgttggtttcgcctggaagtaccgtgcgagcaataaagatgctaagtacagcccgaactggtcacactccaataaagtggaagctgtggtctggacggtacctatcttaatcatcatcttccttgcagtactgacctggaaaaccactcacgctcttgagcctagcaagccgctggcacacgacgagaagcccattaccatcgaagtggtttccatggactggaaatggttcttcatctacccggaacagggcattgctaccgtgaatgaaatcgctttcccggcgaacactccggtgtacttcaaagtgacctccaactccgtgatgaactccttcttcattccgcgtctgggtagccagatttatgccatggccggtatgcagactcgcctgcatctgatcgccaacgaacccggcacttatgacggtatctccgccagctacagcggcccgggcttctcaggcatgaagttcaaagctattgcaacaccggatcgcgccgcattcgaccagtgggtcgcaaaagcgaagcagtcgccgaacaccatgtctgacatggctgcgttcgaaaaactggccgcgcctagcgaatacaaccaggtggaatatttctccaacgtgaaaccagacttgtttgccgatgtaattaacaagtttatggctcacggtaagagcatggacatgacccagccagaaggtgagcacagcgcacacgaaggtatggaaggcatggacatgagccacgcggaatccgcccattaa

SEQ ID NO: 18 - DNA, 72 bp, Escherichia coli
atgagactcaggaaatacaataaaagtttgggatggttgtcattatttgcaggcactgtattgctcagtggc

SEQ ID NO: 19 - DNA, 1524 bp, Escherichia coli
aaaactctggtttattgctcagaaggatctccggaagggtttaacccgcagctgtttacctccggcaccacctatgacgcctcttccgtcccgctttataaccgtctggttgaatttaaaatcggcaccaccgaagtgatcccgggcctcgctgaaaagtgggaagtcagcgaagacggtaaaacctataccttccatctgcgtaaaggtgtgaagtggcacgacaataaagaattcaaaccgacgcgtgaactgaacgccgatgatgtggtgttctcgttcgatcgtcagaaaaacgcgcaaaacccgtaccataaagtttctggcggcagctacgaatacttcgaaggcatgggcttgccagagctgatcagtgaagtgaaaaaggtggacgacaacaccgttcagtttgtgctgactcgcccggaagcgccgttcctcgctgacctggcaatggacttcgcctctattctgtcaaaagaatatgctgatgcgatgatgaaagccggtacaccggaaaaactggacctcaacccaatcggaaccggtccgttccagttacagcagtatcaaaaagattcccgtatccgctacaaagcgtttgatggctactggggcaccaaaccgcagatcgatacgctggttttctctattacccctgacgcttccgtgcgttacgcgaaattgcagaagaatgaatgccaggtgatgccgtacccgaacccggcagatatcgctcgcatgaagcaggataaatccatcaatctgatggaaatgccggggctgaacgtcggttatctctcgtataacgtgcagaaaaaaccactcgatgacgtgaaagttcgccaggctctgacctacgcggtgaacaaagacgcgatcatcaaagcggtttatcagggcgcgggcgtatcagcgaaaaacctgatcccgccaaccatgtggggctataacgacgacgttcaggactacacctacgatcctgaaaaagcgaaagccttgctgaaagaagcgggtctggaaaaaggtttctccatcgacctgtgggcgatgccggtacaacgtccgtataacccgaacgctcgccgcatggcggagatgattcaggcagactgggcgaaagtcggcgtgcaggccaaaattgtcacctacgaatggggtgagtacctcaagcgtgcgaaagatggcgagcaccagacggtaatgatgggctggactggcgataacggggatccggataacttcttcgccaccctgttcagctgcgccgcctctgaacaaggctccaactactcaaaatggtgctacaaaccgtttgaagatctgattcaaccggcgcgtgctaccgacgaccacaataaacgcgttgaactgtacaaacaagcgcaggtggtgatgcacgatcaggctccggcactgatcatcgctcactccaccgtgtttgaaccggtacgtaaagaagttaaaggctatgtggttgatccattaggcaaacatcacttcgaaaacgtctctatcgaataa

SEQ ID NO: 20 - DNA, 84 bp, Escherichia coli
atgcgtatttccttgaaaaagtcagggatgctgaagcttggtctcagcctggtggctatgaccgtcgcagcaagtgttcaggct

SEQ ID NO: 21 - DNA, 84 bp, Escherichia coli
tgcaacaccacgcgtggcgttggtgaagacatttctgatggcggtaacgcgatttctggcgcagcaacgaaagcgcagcaataa

SEQ ID NO: 22 - DNA, 63 bp, Escherichia coli
atggtgaagaagacaattgcagcgatcttttctgttctggtgctttcaacagtattaactgcc

SEQ ID NO: 23 - DNA, 2553 bp, Escherichia coli
gtgaagttcgtaaagtattttttgatccttgcagtctgttgcattctgctgggagcaggctcgatttatggcctataccgctacatcgagccacaactgccggatgtggcgacattaaaagatgttcgcctgcaaattccgatgcagatttacagcgccgatggcgagctgattgctcaatacggtgagaaacgtcgtattccggttacgttggatcaaatcccaccggagatggtgaaagcctttatcgcgacagaagacagccgcttctacgagcatcacggcgttgacccggtggggatcttccgtgcagcaagcgtggcgctgttctccggtcacgcgtcacaaggggcaagtaccattacccagcagctggcgagaaacttcttcctcagtccagaacgcacgctgatgcgtaagattaaggaagtcttcctcgcgattcgcattgaacagctgctgacgaaagacgagatcctcgagctttatctgaacaagatttaccttggttaccgcgcctatggtgtcggtgctgcggcacaagtctatttcggaaaaacggtcgaccaactgacgctgaacgaaatggcggtgatagccgggctgccgaaagcgccttccaccttcaacccgctctactcgatggatcgtgccgtcgcgcggcgtaacgtcgtgctgtcgcggatgctggatgaagggtatatcacccaacaacagttcgatcagacacgcactgaggcgattaacgctaactatcacgcgccggagattgctttctctgcgccgtacctgagcgaaatggtgcgccaggagatgtataaccgttatggcgaaagtgcctatgaagacggttatcgcatttacaccaccatcacccgcaaagtgcagcaggccgcgcagcaggcggtacgtaataacgtgctggactacgacatgcgccacggctatcgcggcccggcaaatgtgctgtggaaagtgggcgagtcggcgtgggataacaacaagattaccgatacgctgaaggcgctgccaacctatggtccgctgctgcctgccgcagtcaccagcgccaatcctcagcaagcgacggcgatgctggcggacgggtcgaccgtcgcattgagtatggaaggcgttcgctgggcgcgtccttaccgttcggatactcagcaaggaccgacgccgcgtaaagtgaccgatgttctgcaaacgggtcagcaaatctgggttcgtcaggttggcgatgcatggtggctggcacaagtgccggaagtgaactcggcgctggtgtcgatcaatccgcaaaacggtgccgttatggcgctggtcggtggctttgatttcaatcagagcaagtttaaccgcgccacccaggcactgcgtcaggtgggttccaacatcaaaccgttcctctacaccgcggcgatggataaaggtctgacgctggcaagtatgttgaacgatgtgccaatttctcgctgggatgcaagtgccggttctgactggcagccgaagaactcaccaccgcagtatgctggtccaattcgcttacgtcaggggctgggtcagtcgaaaaacgtggtgatggtacgcgcaatgcgggcgatgggcgtcgactacgctgcagaatatctgcaacgcttcggcttcccggcacaaaacattgtccacaccgaatcgctggcgctgggttcagcgtccttcaccccaatgcaggtggcgcgcggctacgcggtcatggcgaacggcggcttcctggtggacccgtggtttatcagcaaaattgaaaacgatcagggcggcgtgattttcgaagcgaaaccgaaagtagcctgcccggaatgcgatattccggtgatttacggtgatacgcagaaatcgaacgtgctggaaaataacgatgttgaagatgtcgctatctcccgcgagcagcagaatgtttctgtaccaatgccgcagctggagcaggcaaatcaggcgttagtggcgaagactggcgcgcaggagtacgcaccgcacgtcatcaacactccgctggcattcctgattaagagtgctttgaacaccaatatctttggtgagccaggctggcagggtactggctggcgtgcaggtcgtgatttgcagcgtcgcgatatcggcgggaaaaccgggaccactaacagttcgaaagatgcgtggttctcgggttacggtccgggcgttgtgacctcggtctggattggctttgatgatcaccgtcgtaatctcggtcatacaacggcttccggagcgattaaagatcagatctcaggttacgaaggcggtgccaagagtgcccagcctgcatgggacgcttatatgaaagccgttcttgaaggtgtgccggagcagccgctgacgccgccaccgggtattgtgacggtgaatatcgatcgcagcaccgggcagttagctaatggtggcaacagccgcgaagagtatttcatcgaaggtacgcagccgacacaacaggcagtgcacgaggtgggaacgaccattatcgataatggcgaggcacaggaattgttctga

SEQ ID NO: 24 - DNA, 2535 bp, Escherichia coli
atggccgggaatgaccgcgagccaattggacgcaaagggaaaccgacgcgtccggtcaaacaaaaggtaagccgtcgtcgttacgaagatgacgatgattacgacgattatgatgactatgaggatgaagaaccgatgccgcgcaaaggtaagggcaaaggcaaagggcgtaagcctcgtggcaaacgcggctggctatggctactgctaaaactggctatcgtttttgccgtgctgatcgccatttacggcgtttatctcgatcaaaaaattcgtagccgtattgatggcaaggtctggcaactgcctgcggcagtttatggccgaatggtcaatcttgagccagacatgaccatcagcaagaacgagatggtgaagctgctggaggcgacccagtatcgtcaggtgtcgaaaatgacccgtcctggcgaatttaccgtgcaggccaacagcattgagatgattcgccgtccgtttgatttcccggacagtaaagaaggacaggtgcgcgcgcgtctgacctttgatggcgatcatctggcgacgatcgtcaatatggagaacaaccgtcagttcggtttcttccgtcttgatccgcgtctgatcaccatgatctcttcgccaaacggtgagcagcgtctgtttgtgccgcgcagtggtttcccggatttgctggtggatactttgctggcgacagaagaccgtcatttttacgagcatgatggaatcagtctctactcaatcggacgtgcggtgctggcaaacctgaccgccggacgcacggtacagggtgcgagtacgctgacgcaacagctggtgaaaaacctgttcctctccagcgagcgttcttactggcgtaaagcgaacgaagcttacatggcgctgatcatggacgcgcgttacagcaaagaccgtattcttgagctgtatatgaacgaggtgtatctcggtcagagcggcgacaacgaaatccgcggcttcccgctggcaagcttgtattactttggtcgcccggtagaagagctaagcctcgaccagcaggcgctgttagtcggtatggtgaaaggggcgtccatctacaacccgtggcgtaacccaaaactggcgctggagcgacgtaatctggtgctgcgtctgctgcaacagcaacagattattgatcaagaactctatgacatgttgagtgcccgtccgctgggggttcagccgcgcggtggggtgatctctcctcagccagcctttatgcaactggtgcgtcaggagctgcaggcaaaactgggcgataaggtaaaagatctctccggcgtgaagatcttcactacctttgactcggtggcccaggacgcggcagaaaaagccgccgtggaaggcattccggcactgaagaaacagcgtaagttgagcgatcttgaaactgcgattgtggtcgtcgaccgctttagtggtgaagttcgtgcgatggtcggaggttctgagccgcagtttgcgggctacaaccgtgcgatgcaggcgcgtcgttcgattggttcccttgcaaaaccagcgacttatctgacggccttaagccagccgaaaatctatcgtctgaatacgtggattgcggatgcgccaattgcgctgcgtcagccgaatggccaggtctggtcaccgcagaatgatgaccgtcgttatagcgaaagcggcagagtgatgctggtggatgcgttgacccgttcgatgaacgtgccgacggtaaatctggggatggcgctggggctgcctgcggttacggagacctggattaaactgggcgtaccgaaagatcagttgcatccggttccggcaatgctgctgggggcgttgaacttaacgccaatcgaagtggcgcaggcattccagaccatcgccagcggtggtaaccgtgcaccgctttctgcgctgcgttcggtaatcgcggaagatggcaaagtgctgtatcagagcttcccgcaggcggaacgcgctgttccggcgcaggcggcgtatctgacactatggaccatgcagcaggtggtacaacgcggtacgggtcgtcagcttggggcgaaatacccgaacctgcatctggcagggaaaacagggactaccaacaataacgtagatacctggtttgcgggcattgacggcagcacggtgaccatcacctgggtcggccgtgataacaaccagccgaccaaactgtatggtgccagcggggcaatgtcgatttatcagcgttatctggctaaccagacgccaacgccgctgaatcttgttccgccagaagatattgcagatatgggcgtggactacgacggcaactttgtttgcagcggtggcatgcgtatcttgccggtctggaccagcgatccgcaatcgctgtgccagcagagcgagatgcagcagcagccgtcaggcaatccgtttgatcagtcttctcagccgcagcaacagccgcaacagcaacctgctcagcaagagcagaaagacagcgacggtgtagccggttggatcaaggatatgtttggtagtaattaa

SEQ ID NO: 25 - DNA, 1554 bp, Escherichia coli
gctgatgtacccgcaggcgtcacactggcggaaaaacaaacactggtacgtaacaatggttcagaagttcagtcattagatccgcacaaaattgaaggtgttccggagtctaatatcagccgagacctgtttgaaggcttactggtcagcgatcttgacggtcatccagcacctggcgtcgctgaatcctgggataataaagacgcgaaagtctggaccttccatttgcgtaaagatgcgaaatggtctgatggcacgccagtcacagcacaagactttgtgtatagctggcaacgttctgttgatccgaacactgcttctccgtatgccagttatctgcaatatgggcatatcgccggtattgatgaaattcttgaagggaaaaaaccgattaccgatctcggcgtgaaagctattgatgatcacacattagaagtcaccttaagtgaacccgttccgtacttctataaattacttgttcacccatcaacttcaccggtgccaaaagccgctatcgagaaattcggcgaaaaatggacccagcctggtaatatcgtcaccaacggtgcctataccttaaaagattgggtcgtaaacgaacgaatcgttcttgaacgcagcccgacctactggaacaacgcgaaaaccgttattaaccaggtaacctatttgcctattgcttctgaagttaccgatgtcaaccgctaccgtagtggtgaaatcgacatgacgaataacagcatgccgatcgaattgttccagaagctgaaaaaagagatcccggacgaagttcacgttgatccatacctgtgcacttactattacgaaattaacaaccagaaaccgccattcaacgatgtgcgtgtgcgtaccgcactgaaactaggtatggaccgcgatatcattgttaataaagtgaaagcgcagggcaacatgcccgcctatggttacactccaccgtatactgatggcgcaaaattgactcagccagaatggtttggctggagccaggaaaaacgtaacgaagaagcgaaaaaactgctggctgaagcgggttataccgcagacaaaccgttgaccatcaacctgttgtataacacctccgatctgcataaaaagctggcgattgctgcctcttcattgtggaagaaaaacattggtgtaaacgtcaaactggttaaccaggagtggaaaacgttcctcgacacccgtcaccagggtacttttgatgtggcccgtgcaggctggtgtgctgactacaacgaaccaacttccttcctgaacaccatgctttcgaacagctcgatgaataccgcgcattataagagcccggcctttgacagcattatggcggaaacgctgaaagtgactgacgaggcgcagcgcacagctctgtacactaaagcagaacaacagctggataaggattcggccattgttcctgtttattactacgtgaatgcgcgtctggtgaaaccgtgggttggtggctataccggcaaagatccgctggataatacctatacccggaatatgtacattgtgaagcactaa

SEQ ID NO: 26 - DNA, 78 bp, Escherichia coli
atgaccaacatcaccaagagaagtttagtagcagctggcgttctggctgcgctaatggcagggaatgtcgcgctggca

SEQ ID NO: 27 - DNA, 417 bp, Escherichia coli
tgtgttaataacgacaccctgtcaggggatgtttataccgcttctgaagcgaaacaagtacagaatgtcagctatggcaccatcgttaacgtacgtccggtacagattcagggcggtgatgattccaacgttatcggtgcaattggcggtgctgttcttggtggtttcctggggaatactgttggtggcggaaccgggcgttctctggctactgcagcaggcgctgttgcaggtggcgtagctggtcagggcgtacagagtgcaatgaacaaaacgcagggtgtcgagctggaaattcgtaaagacgatggtaataccatcatggtggtacagaaacaaggcaacactcgtttctctccgggccaacgtgtcgtactggccagcaatggcagtcaggtgaccgtttctccgcgctaa

SEQ ID NO: 28 - DNA, 51 bp, Escherichia coli
atgattaaacgcgtattggttgtttcaatggtaggtctgtctcttgtcggt

SEQ ID NO: 29 - DNA, 693 bp, Escherichia coli
gtgactgacatgaatatccttgatttgttcctgaaggctagccttctggttaaacttatcatgttgattttgattggtttttcaatcgcatcttgggccattattatccagcggacccgtattcttaacgcagcggcgcgcgaagccgaagcgtttgaagataaattctggtctggaatcgaactctctcgcctctatcaagagagccaggggaaacgggataatctgactggttcggaacaaatcttttacagcgggttcaaagagtttgtgcgcctgcatcgtgccaatagccatgcgccggaagccgtagtggaaggggcgtcgcgtgctatgcgtatctccatgaaccgtgaacttgaaaatctggaaacgcacattccgttcctcggtacggttggctccatcagcccgtatattggtctgtttggtacggtctgggggatcatgcacgcctttatcgccctcggggcggtaaaacaagcaacactgcaaatggttgcgcccggtatcgcagaagcgttgattgcgactgcaattggtctgtttgccgctatcccggcagttatggcctacaaccgcctcaaccagcgcgtaaacaaactggaactgaattacgacaactttatggaagagtttaccgcgattctgcaccgccaggcgtttaccgttagcgagagcaacaaggggtaa

SEQ ID NO: 30 - DNA, 429 bp, Escherichia coli
atggccagagcgcgtggacgaggtcgtcgcgatctcaagtccgaaatcaacattgtaccgttgctggacgtactgctggtgctgttgctgatctttatggcgacagcgcccatcatcacccagagcgtggaggtcgatctgccagacgctactgaatcacaggcggtgagcagtaacgataatccgccagtgattgttgaagtgtctggtattggtcagtacaccgtggtggttgagaaagatcgcctggagcgtttaccaccagagcaggtggtggcggaagtgtccagccgtttcaaggccaacccgaaaacggtctttctgatcggtggcgcaaaagatgtgccttacgatgaaataattaaagcactgaacttgttacatagtgcgggtgtgaaatcggttggtttaatgacgcagcctatctaa

SEQ ID NO: 31 - protein, 152 aa, Escherichia coli
CSSNKNASNDGSEGMLGAGTGMDANGGNGNMSSEEQARLQMQQLQQNNIVYFDLDKYDIRSDFAQMLDAHANFLRSNPSYKVTVEGHADERGTPEYNISLGERRANAVKMYLQGKGVSADQISIVSYGKEKPAVLGHDEAAYSKNRRAVLVY

SEQ ID NO: 32 - protein, 21 aa, Escherichia coli
MQLNKVLKGLMIALPVMAIAA

SEQ ID NO: 33 - protein, 137 aa, Escherichia coli
CSAGTGMDANGGNGNMSSEEQARLQMQQLQQNNIVYFDLDKYDIRSDFAQMLDAHANFLRSNPSYKVTVEGHADERGTPEYNISLGERRANAVKMYLQGKGVSADQISIVSYGKEKPAVLGHDEAAYSKNRRAVLVY

SEQ ID NO: 34 - DNA, 414 bp, Escherichia coli
tgttctgccggcactggtatggatgcgaacggcggcaacggcaacatgtcttccgaagagcaggctcgtctgcaaatgcaacagctgcagcagaacaacatcgtttacttcgatctggacaagtacgatatccgttctgacttcgctcaaatgctggatgcacatgcaaacttcctgcgtagcaacccgtcttacaaagtcaccgtagaaggtcacgcggacgaacgtggtactccggaatacaacatctccctgggtgaacgtcgtgcgaacgccgttaagatgtacctgcagggtaaaggcgtttctgcagaccagatctccatcgtttcttacggtaaagaaaaacctgcagtactgggtcatgacgaagcggcatactccaaaaaccgtcgtgcggtactggtttactaa

SEQ ID NO: 35 - protein, 127 aa, Escherichia coli
CSSNKNASNDGSEGMLGALQQNNIVYFDLDKYDIRSDFAQMLDAHANFLRSNPSYKVTVEGHADERGTPEYNISLGERRANAVKMYLQGKGVSADQISIVSYGKEKPAVLGHDEAAYSKNRRAVLVY

SEQ ID NO: 36 - DNA, 384 bp, Escherichia coli
tgttcttccaacaagaacgccagcaatgacggcagcgaaggcatgctgggtgccctgcagcagaacaacatcgtttacttcgatctggacaagtacgatatccgttctgacttcgctcaaatgctggatgcacatgcaaacttcctgcgtagcaacccgtcttacaaagtcaccgtagaaggtcacgcggacgaacgtggtactccggaatacaacatctccctgggtgaacgtcgtgcgaacgccgttaagatgtacctgcagggtaaaggcgtttctgcagaccagatctccatcgtttcttacggtaaagaaaaacctgcagtactgggtcatgacgaagcggcatactccaaaaaccgtcgtgcggtactggtttactaa

SEQ ID NO: 37 - protein, 133 aa, Escherichia coli
CSSNKNASNDGSEGMLGAGTGMDANGGNGNMSSEEQARLQMQQFAQMLDAHANFLRSNPSYKVTVEGHADERGTPEYNISLGERRANAVKMYLQGKGVSADQISIVSYGKEKPAVLGHDEAAYSKNRRAVLVY

SEQ ID NO: 38 - DNA, 402 bp, Escherichia coli
tgttcttccaacaagaacgccagcaatgacggcagcgaaggcatgctgggtgccggcactggtatggatgcgaacggcggcaacggcaacatgtcttccgaagagcaggctcgtctgcaaatgcaacagttcgctcaaatgctggatgcacatgcaaacttcctgcgtagcaacccgtcttacaaagtcaccgtagaaggtcacgcggacgaacgtggtactccggaatacaacatctccctgggtgaacgtcgtgcgaacgccgttaagatgtacctgcagggtaaaggcgtttctgcagaccagatctccatcgtttcttacggtaaagaaaaacctgcagtactgggtcatgacgaagcggcatactccaaaaaccgtcgtgcggtactggtttactaa

SEQ ID NO: 39 - protein, 120 aa, Escherichia coli
CSSNKNASNDGSEGMLGAGTGMDANGGNGNMSSEEQARLQMQQLQQNNIVYFDLDKYDIRSPEYNISLGERRANAVKMYLQGKGVSADQISIVSYGKEKPAVLGHDEAAYSKNRRAVLVY

SEQ ID NO: 40 - DNA, 363 bp, Escherichia coli
tgttcttccaacaagaacgccagcaatgacggcagcgaaggcatgctgggtgccggcactggtatggatgcgaacggcggcaacggcaacatgtcttccgaagagcaggctcgtctgcaaatgcaacagctgcagcagaacaacatcgtttacttcgatctggacaagtacgatatccgttctccggaatacaacatctccctgggtgaacgtcgtgcgaacgccgttaagatgtacctgcagggtaaaggcgtttctgcagaccagatctccatcgtttcttacggtaaagaaaaacctgcagtactgggtcatgacgaagcggcatactccaaaaaccgtcgtgcggtactggtttactaa

SEQ ID NO: 41 - protein, 124 aa, Escherichia coli
CSSNKNASNDGSEGMLGAGTGMDANGGNGNMSSEEQARLQMQQLQQNNIVYFDLDKYDIRSDFAQMLDAHANFLRSNPSYKVTVEGHADERGTISIVSYGKEKPAVLGHDEAAYSKNRRAVLVY

SEQ ID NO: 42 - DNA, 375 bp, Escherichia coli
tgttcttccaacaagaacgccagcaatgacggcagcgaaggcatgctgggtgccggcactggtatggatgcgaacggcggcaacggcaacatgtcttccgaagagcaggctcgtctgcaaatgcaacagctgcagcagaacaacatcgtttacttcgatctggacaagtacgatatccgttctgacttcgctcaaatgctggatgcacatgcaaacttcctgcgtagcaacccgtcttacaaagtcaccgtagaaggtcacgcggacgaacgtggtactatctccatcgtttcttacggtaaagaaaaacctgcagtactgggtcatgacgaagcggcatactccaaaaaccgtcgtgcggtactggtttactaa

SEQ ID NO: 43 - protein, 122 aa, Escherichia coli
CSSNKNASNDGSEGMLGAGTGMDANGGNGNMSSEEQARLQMQQLQQNNIVYFDLDKYDIRSDFAQMLDAHANFLRSNPSYKVTVEGHADERGTPEYNISLGERRANAVKMYLQGKGVSADQI

SEQ ID NO: 44 - DNA, 369 bp, Escherichia coli
tgttcttccaacaagaacgccagcaatgacggcagcgaaggcatgctgggtgccggcactggtatggatgcgaacggcggcaacggcaacatgtcttccgaagagcaggctcgtctgcaaatgcaacagctgcagcagaacaacatcgtttacttcgatctggacaagtacgatatccgttctgacttcgctcaaatgctggatgcacatgcaaacttcctgcgtagcaacccgtcttacaaagtcaccgtagaaggtcacgcggacgaacgtggtactccggaatacaacatctccctgggtgaacgtcgtgcgaacgccgttaagatgtacctgcagggtaaaggcgtttctgcagaccagatctaa

SEQ ID NO: 45 - protein, 148 aa, Escherichia coli
CSSNKNASNDGSEGMLGAGTGMDANGGNGNMSSEEQARLQMQQLQQNNIVYFDLDKYDIRSDFAQMLDAHANFLRSNPSYKVTVEGHADERGTPEYNISLGERRANAVKMYLQGKGVSADQISIVEKPAVLGHDEAAYSKNRRAVLVY

SEQ ID NO: 46 - DNA, 447 bp, Escherichia coli
tgttcttccaacaagaacgccagcaatgacggcagcgaaggcatgctgggtgccggcactggtatggatgcgaacggcggcaacggcaacatgtcttccgaagagcaggctcgtctgcaaatgcaacagctgcagcagaacaacatcgtttacttcgatctggacaagtacgatatccgttctgacttcgctcaaatgctggatgcacatgcaaacttcctgcgtagcaacccgtcttacaaagtcaccgtagaaggtcacgcggacgaacgtggtactccggaatacaacatctccctgggtgaacgtcgtgcgaacgccgttaagatgtacctgcagggtaaaggcgtttctgcagaccagatctccatcgttgaaaaacctgcagtactgggtcatgacgaagcggcatactccaaaaaccgtcgtgcggtactggtttactaa

SEQ ID NO: 47 - protein, 148 aa, Escherichia coli
CSSNKNASNDGSEGMLGAGTGMDANGGNGNMSSEEQARLQMQQLQQNNIVYFDLDKYDIRSDFAQMLDAHANFLRSNPSYKVTVEGHADERGTPEYNISLGERRANAVKMYLQGKGVSADQISIVSYGKEKPAVLGHDEAAYSAVLVY

SEQ ID NO: 48 - DNA, 447 bp, Escherichia coli
tgttcttccaacaagaacgccagcaatgacggcagcgaaggcatgctgggtgccggcactggtatggatgcgaacggcggcaacggcaacatgtcttccgaagagcaggctcgtctgcaaatgcaacagctgcagcagaacaacatcgtttacttcgatctggacaagtacgatatccgttctgacttcgctcaaatgctggatgcacatgcaaacttcctgcgtagcaacccgtcttacaaagtcaccgtagaaggtcacgcggacgaacgtggtactccggaatacaacatctccctgggtgaacgtcgtgcgaacgccgttaagatgtacctgcagggtaaaggcgtttctgcagaccagatctccatcgtttcttacggtaaagaaaaacctgcagtactgggtcatgacgaagcggcatactccgcggtactggtttactaa

SEQ ID NO: 49 - protein, 58 aa, Escherichia coli
CSSNAKIDQLSSDVQTLNAKVDQLSNDVNAMRSDVQAAKDDAARANQRLDNMATKYRK

SEQ ID NO: 50 - protein, 325 aa, Escherichia coli
APKDNTWYTGAKLGWSQYHDTGFINNNGPTHENQLGAGAFGGYQVNPYVGFEMGYDWLGRMPYKGSVENGAYKAQGVQLTAKLGYPITDDLDIYTRLGGMVWRADTKSNVYGKNHDTGVSPVFAGGVEYAITPEIATRLEYQWTNNIGDAHTIGTRPDNGMLSLGVSYRFGQGEAAPVVAPAPAPAPEVQTKHFTLKSDVLFNFNKATLKPEGQAALDQLYSQLSNLDPKDGSVVVLGYTDRIGSDAYNQGLSERRAQSVVDYLISKGIPADKISARGMGESNPVTGNTCDNVKQRAALIDCLAPDRRVEIEVKGIKDVVTQPQA

SEQ ID NO: 51 - protein, 421 aa, Escherichia coli
MSKATEQNDKLKRAIIISAVLHVILFAALIWSSFDENIEASAGGGGGSSIDAVMVDSGAVVEQYKRMQSQESSAKRSDEQRKMKEQQAAEELREKQAAEQERLKQLEKERLAAQEQKKQAEEAAKQAELKQKQAEEAAAKAAADAKAKAEADAKAAEEAAKKAAADAKKKAEAEAAKAAAEAQKKAEAAAAALKKKAEAAEAAAAEARKKAATEAAEKAKAEAEKKAAAEKAAADKKAAAEKAAADKKAAEKAAAEKAAADKKAAAEKAAADKKAAAAKAAAEKAAAAKAAAEADDIFGELSSGKNAPKTGGGAKGNNASPAGSGNTKNNGASGADINNYAGQIKSAIESKFYDASSYAGKTCTLRIKLAPDGMLLDIKPEGGDPALCQAALAAAKLAKIPKPPSQAVYEVFKNAPLDFKP

SEQ ID NO: 52 - protein, 25 aa, Escherichia coli
GTGMDANGGNGNMSSEEQARLQMQQ

SEQ ID NO: 53 - protein, 4 aa, Escherichia coli
SKNR

SEQ ID NO: 54 - DNA, 849 bp, Escherichia coli
gtaacttatcctctgccaaccgacgggagtcgcctggttggtcagaatcaggtgatcaccattcctgaaggtaacactcagccgctggagtattttgccgccgagtaccagatggggctttccaatatgatggaagcgaacccgggtgtggataccttcctgccgaaaggcggtactgtactgaacattccgcagcagctgatcctgccggataccgttcatgaaggcatcgtcattaacagtgctgagatgcgtctttattactatccgaaagggaccaacaccgttatcgtgctgccgatcggcattggtcagttaggcaaagatacgcctatcaactggaccaccaaagttgagcgtaaaaaagcaggcccgacctggacgccgaccgccaaaatgcacgcagagtaccgcgctgcgggcgaaccgcttccggctgtcgttccggcaggtccggataacccgatggggctgtatgcactctatatcggtcgcctgtatgctatccatggcaccaacgccaacttcggtatcggcctgcgtgtaagtcatggttgtgtgcgtctgcgtaacgaagacatcaaattcctgttcgagaaagtaccggtcggtacccgcgtacagtttattgatgagccggtaaaagcgaccaccgagccagacggcagccgttatattgaagtccataacccgctgtctaccaccgaagcccagtttgaaggtcaggaaattgtgccaattaccctgacgaagagcgtgcagacagtgaccggtcagccagatgttgaccaggttgttcttgatgaagcgattaaaaaccgctccgggatgccggttcgtctgaattaa

SEQ ID NO: 55 - DNA, 72 bp, Escherichia coli
atgaatatgaaattgaaaacattattcgcagcggccttcgctgttgtcggcttttgcagtaccgcctctgcg

SEQ ID NO: 56 - DNA, 894 bp, Escherichia coli
ctaccggcaaaagccaacacctggccgctgccgccagcgggcagtcgtctggttggcgaaaacaaatttcatgtggtggaaaatgacggtggttctctggaagccatcgccaaaaaatacaacgtcggctttctcgctctgttacaggctaaccccggcgttgatccttacgtaccgcgcgcgggcagcgtgttaacgatcccgttgcaaaccctacttccagatgcgccgcgcgaaggcattgtgatcaacattgcggagctgcgtctctattactacccgccgggtaaaaattcggtaaccgtgtatccaataggtattggtcagttaggtggtgacacgctgacaccgacaatggtgaccaccgtttcagacaaacgtgcaaacccaacctggacgccaacggcaaacatccgcgcccgttataaagcacagggaattgagttgcctgcggtagtgccggctggactggataacccaatgggccatcatgcgattcgtctggcggcctatggcggcgtttatttgcttcatggtacgaacgccgatttcggcattggcatgcgggtaagttctggctgtattcgtctgcgggatgacgatatcaaaacactctttagccaggtcaccccaggcaccaaagtgaatatcatcaacactccgataaaagtctctgccgaaccaaacggtgcgcgtctggttgaagtacatcagccgctgtcagagaagattgatgacgatccgcagctgctgccaattacgctgaatagcgcaatgcaatcatttaaagatgcagcacaaactgacgctgaagtgatgcaacatgtgatggatgtccgttccgggatgccggtggatgtccgccgtcatcaagtgagcccacaaacgctgtaa

SEQ ID NO: 57 - DNA, 69 bp, Escherichia coli
gtgatgatcaaaacgcgtttttctcgctggctaacgttttttacgttcgccgctgccgtggcgctggcg

SEQ ID NO: 58 - DNA, 870 bp, Escherichia coli
gtaacttatccattacctccagagggtagccgtttagtggggcagtcgtttactgtaactgttcctgatcacaatacccagccgctggagacttttgccgcacaatacgggcaagggttaagtaacatgctggaagcgaacccgggcgctgatgtttttttgccgaagtctggctcgcaactcaccattccgcagcaactgattttgcccgacactgttcgtaaagggattgttgttaacgtcgctgagatgcgtctttattactacccaccagacagtaatactgtggaagtctttcctattggtatcggccaggctgggcgagaaaccccgcgtaactgggtgactaccgttgaacgtaaacaagaagctccaacctggacgccaacgccgaacactcggcgcgaatatgcgaaacgaggggagagtttgcccgcatttgttcctgcgggccccgataatcccatggggctgtacgcgatttatattggcaggttgtatgccatccatggtaccaatgccaattttggtattgggctccgggtaagtcagggctgtattcgtctgcgcaatgacgatatcaaatatctgtttgataatgttcctgttgggacgcgtgtgcaaattatcgaccagccagtaaaatacaccactgaaccagatggctcgaactggctggaagttcatgagccattgtcgcgcaatcgtgcagaatatgagtctgaccgaaaagtgccattgccggtaaccccatctttgcgggcgtttatcaacgggcaagaagttgatgtaaatcgcgcaaatgctgcgttgcaacgtcgatcgggaatgcctgtgcaaattagttctggttcaagacagatgttttaa

SEQ ID NO: 59 - DNA, 63 bp, Escherichia coli
atgcgtcgtgtaaatattctttgctcatttgctctgctttttgccagccatactagcctggcg

SEQ ID NO: 60 - protein, 20 aa, Escherichia coli
MKATKLVLGAVILGSTLLAG

SEQ ID NO: 61 - protein, 21 aa, Escherichia coli
MKKTAIAIAVALAGFATVAQA

SEQ ID NO: 62 - DNA, 2373 bp, Escherichia coli
gctgaagggttcgtagtgaaagatattcatttcgaaggccttcagcgtgtcgccgttggtgcggccctcctcagtatgccggtgcgcacaggcgacacggttaatgatgaagatatcagtaataccattcgcgctctgtttgctaccggcaactttgaggatgttcgcgtccttcgtgatggtgatacccttctggttcaggtaaaagaacgtccgaccattgccagcattactttctccggtaacaaatcggtgaaagatgacatgctgaagcaaaacctcgaggcttctggtgtgcgtgtgggcgaatccctcgatcgcaccaccattgccgatatcgagaaaggtctggaagacttctactacagcgtcggtaaatatagcgccagcgtaaaagctgtcgtgaccccgctgccgcgcaaccgtgttgacctaaaactggtgttccaggaaggtgtgtcagctgaaatccagcaaattaacattgttggtaaccatgctttcaccaccgacgaactgatctctcatttccaactgcgtgacgaagtgccgtggtggaacgtggtaggcgatcgtaaataccagaaacagaaactggcgggcgaccttgaaaccctgcgcagctactatctggatcgcggttatgcccgtttcaacatcgactctacccaggtcagtctgacgccagataaaaaaggtatttacgtcacggtgaacatcaccgaaggcgatcagtacaagctttctggcgttgaagtgagcggcaaccttgccgggcactccgctgaaattgagcagctgactaagatcgagccgggtgagctgtataacggcaccaaagtgaccaagatggaagatgacatcaaaaagcttctcggtcgctatggttatgcctatccgcgcgtacagtcgatgcccgaaattaacgatgccgacaaaaccgttaaattacgtgtgaacgttgatgcgggtaaccgtttctacgtgcgtaagatccgttttgaaggtaacgatacctcgaaagatgccgtcctgcgtcgcgaaatgcgtcagatggaaggtgcatggctggggagcgatctggtcgatcagggtaaggagcgtctgaatcgtctgggcttctttgaaactgtcgataccgatacccaacgtgttccgggtagcccggaccaggttgatgtcgtctacaaggtaaaagagcgcaacaccggtagcttcaactttggtattggttacggtactgaaagtggcgtgagcttccaggctggtgtgcagcaggataactggttaggtacaggttatgctgttggtatcaacgggaccaaaaacgattaccagacctatgctgaactgtcggtaaccaacccgtacttcaccgtagatggcgtaagcctcggtggtcgtctcttctataatgacttccaggcagatgacgccgacctgtccgactataccaacaagagttatggtacagacgtgacgttgggcttcccgattaacgaatataactcgctgcgtgcaggtctgggttatgtacataactccctgtccaacatgcagcctcaggttgcgatgtggcgttatctgtactctatgggtgaacatccgagcacctctgatcaggataacagcttcaaaacggacgacttcacgttcaactatggttggacctataacaagcttgaccgtggttacttcccgacagatggttcacgtgtcaacctgaccggtaaagtgaccattcctggatcggataacgaatactacaaagtgacgttagacacggcgacttatgtgccgatcgatgacgatcacaaatgggttgttctggggcgtacccgctggggttatggtgatggtttaggcggcaaagagatgccgttctacgagaacttctatgccggtggttccagcaccgtgcgtggcttccagtccaataccattggtccgaaagcagtttacttcccgcatcaggccagtaattatgatccggactatgattacgaatgtgcgactcaggacggcgcgaaagacctgtgtaaatcggatgatgctgtaggcggtaacgccatggcggttgccagcctcgagttcatcaccccgacgccgtttattagcgataagtatgctaactcggttcgtacttccttcttctgggatatgggtaccgtttgggatacaaactgggattccagccaatattctggatatccggactatagtgatccaagcaatatccgtatgtctgcgggtatcgcattacaatggatgtccccattggggccgttggtgttctcctacgcccagccgttcaaaaagtacgatggagacaaggcagaacagttccagtttaacatcggtaaaacctggtaa

SEQ ID NO: 63 - DNA, 60 bp, Escherichia coli
atggcgatgaaaaagttgctcatagcgtcgctgctgtttagcagcgccaccgtatacggt

SEQ ID NO: 64 - DNA, 549 bp, Escherichia coli
gatgccgcaagcgatctgaaaagccgcctggataaagtcagcagcttccacgccagcttcacacaaaaagtgactgacggtagcggcgcggcggtgcaggaaggtcagggcgatctgtgggtgaaacgtccaaacttattcaactggcatatgacacaacctgatgaaagcattctggtttctgacggtaaaacactgtggttctataacccgttcgttgagcaagctacggcaacctggctgaaagatgccaccggtaatacgccgtttatgctgattgcccgcaaccagtccagcgactggcagcagtacaatatcaaacagaatggcgatgactttgtcctgacgccgaaagccagcaatggcaatctgaagcagttcaccattaacgtgggacgtgatggcacaatccatcagtttagcgcggtggagcaggacgatcagcgcagcagttatcaactgaaatcccagcaaaatggggctgtggatgcagcgaaatttaccttcaccccgccgcaaggcgtcacggtagatgatcaacgtaagtag

SEQ ID NO: 65 - DNA, 63 bp, Escherichia coli
atgaaaaaaattgccatcacctgtgcattactctcaagcttagtagcaagcagcgtttgggct

SEQ ID NO: 66 - DNA, 561 bp, Escherichia coli
tgttccgttaccacgcccaaaggtcctggcaaaagcccggattcgccacaatggcgtcagcatcagcaagacgtgcgcaatcttaatcagtatcagactcgcggcgcgttcgcttatatttctgaccaacaaaaagtgtacgcccgctttttctggcagcaaaccggccaggatcgctaccgtctgctgctcactaacccattgggcagcacggaactggagctgaatgctcaaccgggtaacgtgcagttagtcgacaataaaggtcagcgttataccgccgatgacgccgaagagatgattggcaaattgaccggaatgccaattccgctcaacagcttgcgccagtggattttaggtttaccgggtgatgcaaccgactacaaactggacgaccagtaccgcctgagcgaaattacctacagccagaatggcaaaaactggaaggttgtttatggtggttatgacaccaaaacgcaacctgcgatgccagccaatatggaactcaccgacggtggtcaacgcatcaagttaaaaatggataactggatagtgaaataa

SEQ ID NO: 67 - DNA, 63 bp, Escherichia coli
atgcccctgcccgattttcgtcttatccgcctgctaccgctggctgctcttgtgctcactgcc

SEQ ID NO: 68 - DNA, 1200 bp, Escherichia coli
atgtaccaacctgtcgctctatttattggcctgcgttacatgcgtgggcgtgcagcggatcgcttcggtcgtttcgtctcctggctttctaccatcggcattaccctcggggtgatggcgctggtcacagtattgtcagtgatgaacggctttgagcgcgagctgcaaaacaacatccttggcctgatgccacaggcaattctctcttctgagcatggctctcttaacccgcagcaactcccagaaacggcagtcaaactggacggcgttaatcgcgtcgcacctattactaccggtgatgtggtactgcaaagcgcgcgcagcgtggcggtcggggtgatgctcggtatcgacccggcgcaaaaagatccacttacaccgtatctggtcaatgtgaaacaaactgacctcgagccggggaaatataatgtcatcctcggcgaacaacttgcctcacagctaggcgttaatcgcggtgatcaaatccgcgtgatggtaccatctgccagccagttcacgccgatggggcgtattccaagccagcgcctgttcaatgtgattggcactttcgccgccaacagtgaagtcgatggctatgaaatgctggtgaatattgaggatgcctcgcgtctgatgcgttatccggcaggcaatattaccggctggcgtttgtggctggatgagccgctgaaagtcgactcattaagtcagcaaaaactgcctgaaggcagcaaatggcaggactggcgtgatcgtaaaggcgagttgttccaggccgtacgcatggaaaaaaatatgatgggtttactgctgagcctgattgtcgccgttgcggcgtttaacattattacctcactagggctgatggtaatggagaagcagggcgaagtagcgatcctgcaaacgcaaggcttaactccgcgacaaatcatgatggtctttatggtgcaaggggccagcgccgggattatcggtgcgatcctcggagcggcgcttggcgccctgcttgccagccagttaaataatctgatgccgataatcggcgtcctgcttgatggcgcggcgctgccggtggctatcgaacctttacaggtcattgttattgcgctggtggcgatggctatcgcgctgctgtctacgctttacccttcatggcgcgctgccgccactcaacccgctgaggctttacgttatgaataa

SEQ ID NO: 69 - DNA, 702 bp, Escherichia coli
atgaataagatcctgttgcaatgcgacaacctgtgcaaacgctatcaggaaggcagtgtgcaaaccgatgtgctgcacaatgtcagtttcagcgtcggcgaaggtgaaatgatggcgatcgtcggtagctctggttccggtaaaagtaccttgctgcacctgctgggcgggctggatacgccaacctccggcgatgtgatttttaatggtcagccaatgagcaaactgtcgtcggcagcgaaagctgaactgcgcaaccagaagctgggctttatttatcagtttcaccacctgctgccggattttaccgccctggaaaacgtggctatgccgctgctgattggcaagaaaaagcccgctgaaatcaacagccgtgcacttgagatgttaaaagcggtggggctggatcatcgtgcgaatcaccgcccatctgaactttctggcggcgaacgccagcgtgtggcgattgcccgtgcgctggtgaataacccgcgcctggtactggcggatgaacctaccggtaacctcgatgcgcgtaacgccgacagcatcttccagttgcttggggaattgaatcgcttgcagggcaccgccttcctggtggttactcacgacctgcaactggcgaaacgtatgagccgccagttagaaatgcgtgatggtcgtctgacggcggaactgagcctgatgggggcggagtaa

SEQ ID NO: 70 - DNA, 1245 bp, Escherichia coli
atggcgatgcctttatcgttattaattggcctgcgttttagtcgcggacggcggcgcggcggcatggtgtcgctgatctccgttatttctaccattggcattgccctcggcgtggcggtattgatcgtcggcttaagcgcgatgaacggctttgaacgcgaactgaacaaccgtattctggcggtggtgccgcatggtgaaatcgaggcggtggatcagccgtggactaactggcaggaagcactggatcacgtgcaaaaagtgccgggtattgccgctgccgcgccgtatatcaatttcaccgggctggtggaaagtggcgcgaatcttcgcgcaatccaggtgaagggcgttaacccgcaacaggaacagcgtctgagcgcattaccctcgtttgtccagggcgatgcgtggcgcaattttaaagcgggcgaacagcaaattatcatcggcaaaggcgtggcggatgcgctgaaagtgaagcagggggattgggtgtcgattatgatccccaactcgaatcccgagcataaactgatgcagccaaaacgtgtgcgtttgcacgttgccggtattttgcagttgagtggtcaactcgatcacagttttgccatgatcccgctggcggatgcccaacaatatcttgatatgggttccagcgtgtcaggtattgcccttaaaatgacggatgttttcaacgccaataagctggtacgcgatgcgggtgaagtgaccaacagctatgtttatattaaaagctggattggtacttacggctatatgtatcgcgatatccaaatgatccgcgccattatgtatctggcgatggtactggtgattggcgtggcctgtttcaacatcgtctccaccttagtgatggcggtgaaagacaagagtggcgatatcgcagtattaagaacgctgggggcgaaagatggtttaattcgcgccatctttgtctggtatggattgctggcagggctgttcggcagcctgtgtggtgtgattatcggcgtagtggtttcactgcaacttaccccgattattgagtggattgaaaagttgatcggtcatcagttcctctccagcgatatctattttattgatttcctgccatcggaattgcactggctggacgtcttctacgtactggtcacagcattgttgctgagtcttttggcaagttggtatccggcgcggcgcgccagtaatattgaccctgcgcgagtccttagcggccagtaa

SEQ ID NO: 71 - DNA, 528 bp, Escherichia coli
tgtggctggcatctgcgtgataccacgcaggttccttccactatgaaggtcatgatcctggactcaggcgatccgaacgggccattaagccgtgcggtgcgtaaccagttacgtctgaatggtgtcgagttgcttgataaagaaaccacgcgtaaggacgttccatccttgcgtttgggtaaagtgagcatcgcgaaagataccgcatcggtattccgtaacggtcaaacagcagagtatcagatgatcatgacggttaatgcgaccgtgttgatccccggccgtgatatctacccgattagcgccaaagtcttccgttcgttcttcgataacccgcaaatggcgttagcgaaagataacgaacaagacatgatcgtaaaagagatgtacgaccgtgctgccgaacagctgattcgtaagctgccaagcatccgtgctgcggatattcgttccgacgaagaacagacgtcgaccacaacggatactccggcaacgcctgcacgcgtctccaccacgctgggtaactga

SEQ ID NO: 72 - DNA, 54 bp, Escherichia coli
gtgcgatatctggcaacattgttgttatctctggcggtgttaatcaccgccggg

SEQ ID NO: 73 - DNA, 2283 bp, Escherichia coli
gccgacctcgcctcacagtgcatgttgggcgtgccaagctatgaccgtcctctggtacagggcgataccaatgacttacccgtgactatcaatgctgaccacgcgaaaggggactacccggatgacgccgtgtttactggcagcgtggatatcatgcagggtaacagccgtctgcaggccgacgaagtgcagctccatcaaaaagaggcaccaggacaaccggagccggtacgtaccgttgatgcgctcggtaatgtccattacgacgataaccaggtgatcctcaaagggccgaaaggctgggcgaatctgaacaccaaagataccaacgtctgggaaggtgattaccagatggtgggtcgccagggtcgcggtaaagcggacctgatgaaacaacgtggcgaaaaccgctataccattctggataacggtagctttacctcctgtctgccgggttctgacacctggagcgtggtaggtagcgaaattattcatgaccgcgaagaacaagttgcggagatctggaacgcccgctttaaggtgggtccggtaccgatcttttatagcccctatttgcagttgccggtgggtgacaaacgtcgctctggtttcttgatcccgaacgccaagtacaccaccaccaactactttgagttctacctgccatattactggaacatcgcgccaaatatggatgccaccatcacgccgcattatatgcatcgtcgtggcaacatcatgtgggagaacgaattccgctacctctcccaggcgggcgctggcttgatggaactggactatctgccttcagataaagtctatgaagatgaacacccgaacgatgacagttcacgtcgttggttattctactggaaccactccggggtcatggatcaggtgtggcgtttcaacgtcgactacaccaaggtcagcgatcctagctacttcaatgatttcgataacaagtacggttccagtactgacggctacgcaacgcaaaaattcagcgttggctatgcggtgcaaaacttcaatgccaccgtttcaaccaagcagttccaggttttcagcgaacagaacaccagtagctactcggcagagccgcagttagacgttaattactaccagaatgatgttggtccgtttgatacgcgtatttacggccaggcagtgcactttgttaacaccagagacgacatgcctgaagcaacccgtgttcacctggaaccgaccatcaatttgccgctctctaataactggggcagcatcaataccgaagcgaagttgctggcaacccattatcagcaaaccaatcttgactggtataactccagaaacacgaccaagctggacgaatccgttaaccgcgtaatgccgcaattcaaagttgacggcaaaatggtctttgaacgcgatatggaaatgctggctccgggttatacccaaacgctggaaccgcgcgcgcagtatttgtacgtgccgtatcgcgatcagagcgacatctataactacgactcgtctctgctgcaatctgactactctggcctgttccgggaccggacttacggcggtcttgaccgtattgcctccgctaaccaggtgacgaccggtgtcacatctcgcatatatgatgatgctgccgttgaacgttttaatatttccgttggtcaaatctactatttcacggagtctcgcactggcgatgacaacataacatgggagaatgacgacaaaacgggttcactggtgtgggcaggcgatacttactggcgtatctccgagcgttggggattgcgtggcgggattcagtacgatacacgtctggataacgtagcgaccagtaactccagcattgaataccgtcgggatgaagaccgtctggtacagctgaattaccgttacgccagcccggaatatattcaggctacgctgcctaagtactattccactgctgagcaatataagaatggtatttcgcaggtaggtgctgtcgccagctggccaattgccgatcgttggtccattgttggggcctactactacgacaccaatgctaacaagcaagccgactctatgttaggtgtgcaatacagctcctgctgctatgcaattcgcgtcggttacgagcggaagctgaacggttgggataacgataaacaacatgcggtatatgacaacgcaatcggctttaacatcgaacttcgcggcctgagctccaactacggtctgggtacgcaagagatgctgcgttcgaacattctgccgtatcaaaacactttgtga

SEQ ID NO: 74 - DNA, 72 bp, Escherichia coli
atgaaaaaacgtatccccactctcctggccaccatgattgccaccgccctttatagtcaacagggactggca

SEQ ID NO: 75 - DNA, 477 bp, Escherichia coli
gtaaccggagacactgatcagccgatccacattgaatcggaccagcaatctcttgatatgcaaggcaacgtggttacctttaccggtaatgtcatcgtcacccagggcaccatcaaaattaatgccgacaaagtggtcgttacccgtccgggcggcgaacaaggtaaagaagtgattgacggctacggtaaaccggcaacgttctaccagatgcaggacaacggtaaacccgttgaaggtcacgcttcccagatgcactacgaactggcaaaagattttgtcgttctgacgggtaatgcttatctgcagcaggtcgatagcaacattaagggcgataagatcacttacctggtgaaagagcagaaaatgcaggctttcagcgacaaaggcaagcgcgtaacaaccgttctggtgccgtcgcagctgcaggacaaaaacaacaaaggccagaccccggcacagaagaagggtaattaa

SEQ ID NO: 76 - DNA, 81 bp, Escherichia coli
atgaaattcaaaacaaacaaactcagccttaatcttgtgcttgccagctcacttctggccgccagcattccggcatttgcc

SEQ ID NO: 77 - DNA, 726 bp, Escherichia coli
atggcaacattaactgcaaagaaccttgcaaaagcctataaaggccgtcgcgtggtagaagacgtcagcctgaccgtcaactccggggaaattgtcggtctgctggggccaaacggtgccggtaagaccaccactttctacatggttgtaggcattgtgccgcgcgatgcgggcaacatcattattgatgatgacgatatcagtctgctgcctctgcatgcacgcgcgcgccgcggtatcggctatctgccacaggaagcctccattttccgtcgcctcagcgtttacgataacctgatggcggtactgcaaattcgtgacgacttgtctgctgaacaacgtgaagaccgcgcgaacgagctgatggaagagtttcacattgagcacctgcgtgacagcatggggcagtcactctccgggggtgaacgtcgccgtgtagaaattgcccgcgcactggctgcgaatccgaaatttattctgctcgacgaaccgtttgccggggttgacccgatctcggttatcgacattaaacgcatcattgagcacctgcgcgacagcggcctgggcgtgctgatcactgaccacaacgtgcgtgaaacactggcggtttgtgaacgcgcttatatcgtcagtcaggggcatttgatcgcccacggcacgcctacagaaatcttacaagacgaacacgttaagcgtgtataccttggggaagacttcagactctga

SEQ ID NO: 78 - DNA, 1100 bp, Escherichia coli
gtgataatcataagatatctggtgcgggagacgctcaaaagccagctggcgatactcttcatcttgcttttgatcttcttctgtcaaaagttagtgaggatcctcggcgcagcggttgacggcgatattccggcgaatctggtgctctcccttctcgggttgggcgtgccggaaatggcgcagcttatcctgccattaagcctgttcctcgggctgctgatgacgctgggcaaactgtataccgaaagtgaaattacggtaatgcatgcctgcggcctgagcaaagcggttctggtgaaagcggcaatgatccttgcggtattcacggcaatcgtagcggcggttaacgtgatgtgggcgggaccgtggtcatcgcgtcatcaggatgaagtgttagcagaagcgaaagcgaaccctggcatggcggcgctggcgcaagggcaattccagcaagcgactaatggcagctcggtgctgttcatcgaaagcgttgacggcagcgatttcaaagatgtgttcctcgcgcaaattcgaccaaaaggtaatgcacgtccttctgtggtggtggccgattccggacatttaacccagctgcgcgacggctcccaggtcgtcactctcaaccagggaacgcgcttcgaaggcactgcattgttacgtgatttccgcattacggacttccaggattatcaggcgatcattggtcaccaggcggtggcgctcgacccgaacgataccgaccagatggacatgcgcacattgtggaacactgacaccgatcgtgctcgcgcagaactgaactggcgtatcacgttggtattcaccgtgtttatgatggcacttatggtcgtaccgctgagcgtggttaacccacgtcagggacgcgtactgtcgatgctgccagccatgctgctgtatctacttttcttcctgatccagacctccctgaaatcgaacggcggtaaaggtaagctggacccgacgctgtggatgtggaccgttaacctgatttatctggctttagcgattgttctcaacctttgggacaccgtgccggtccgccgcctgcgcgccagtttttcgcgtaaaggagcggtgtg

SEQ ID NO: 79 - DNA, 1083 bp, Escherichia coli
atgcaaccttttggcgtacttgaccgctatatcggtaaaactattttcaccaccatcatgatgacactgttcatgctggtgtcgctgtcgggcattatcaagtttgtcgatcagctgaaaaaagccgggcaggggagttacgacgcgttaggcgcaggaatgtataccttgctgagcgtgccgaaagatgtgcagatcttcttcccgatggcggctctgcttggggcgttgcttggtcttgggatgctggcgcagcgcagcgaactggtggtgatgcaggcttctggttttacccgtatgcaggtggcgctgtcggtgatgaaaaccgccattccgctggtcttgctgacgatggcgattggcgaatgggtcgcgccgcagggcgagcagatggcgcgtaactaccgtgcgcaggcgatgtacggcggctcgttgctctctacccagcaaggcttatgggcgaaagatggcaacaacttcgtctacattgagcgggttaaaggtgacgaagagttaggtggcatcagcatttatgcctttaacgagaatcgtcgtctgcaatccgtacgctatgccgctactgcgaagtttgacccggaacataaagtctggcgtctgtcgcaggttgatgaatctgatctgaccaatccgaaacagattaccggttcgcagacggtgagcggcacctggaaaaccaacctcacgccggacaaactgggcgtggtggcgctggacccggatgcactctctatcagcggtttgcacaactatgtgaagtatctgaagtcgagcggtcaggatgccggacgttatcagctcaacatgtggagcaaaatcttccagccgctatctgtggcggtgatgatgctgatggcgctgtcgttcatctttggcccactgcgtagcgtaccgatgggcgtgcgtgtggtcaccggtatcagtttcggttttgtcttctacgtactggaccagatcttcggcccgctgacgttggtttatggcatcccgccgatcatcggcgcactgttgccaagcgccagcttcttcttaatcagcctgtggctgttaatgagaaaatcgtaa

SEQ ID NO: 80 - DNA, 1959 bp, Escherichia coli
tgtggcacccatactcccgatcagtccactgcttatatgcagggcacggcgcaggctgattctgccttttatcttcagcagatgcagcaaagctctgatgataccaggatcaactggcaattactcgccattcgtgcactggtgaaagaaggtaaaaccgggcaggcggttgagttgtttaaccaactaccgcaagaactgaacgatgctcagcgtcgcgagaaaacactgctggcggtagagattaaactggcgcagaaagattttgctggcgcgcaaaacttgctggcgaaaatcacacctgccgatttagaacaaaaccagcaagcgcgttactggcaggcaaaaatcgatgccagccaggggcgtccttccattgatttactgcgcgcgttaattgctcaggaaccgctgcttggcgcgaaagaaaaacagcagaatattgatgccacctggcaggcgctctcctccatgactcaggaacaggcgaatacgctggtgatcaacgccgacgaaaatattctgcaaggctggctggatctgcagcgcgtctggtttgataaccgtaacgatcccgacatgatgaaagccgggatcgccgactggcagaaacgttatccgaacaatccgggcgcgaaaatgctgccaacgcagttggttaacgtaaaagcgtttaaaccagcctcgaccaacaaaatcgccctgctgttgccactgaatggccaggcagcggtatttggtcgcactattcagcaaggctttgaagcggcgaaaaatatcggcactcagccagtggcagctcaggtagctgccgcacctgccgcagacgtagctgaacaacctcagccgcaaaccgtggatggcgttgccagcccggcacaagcctcggttagcgatctgaccggtgaacagcctgcagcccagccggtgcctgtaagcgccccggcgacaagcaccgcagcggtaagcgcacccgcaaatccatccgcagagctgaaaatctacgatacctcatcacaaccacttagccagatcttaagccaggttcagcaggatggcgcgagtattgtggtcggtccgttgctgaaaaataacgttgaagagttgctgaagagcaacactccgctgaacgtactggcactgaaccagccggagaatatcgaaaatcgcgtcaatatttgttacttcgcgctttcaccggaagacgaagcgcgcgatgcagcgcgtcatattcgtgaccagggtaaacaagcgccgctggtgctgatcccacgcagttcattgggcgatcgcgtagccaatgcgtttgcgcaagagtggcagaaactgggcggcggcaccgttctgcaacaaaaatttggttccaccagcgaattacgcgcgggtgttaacggcggttctggtattgctttaacgggtagcccgattactctcagagcgacaaccgactccggcatgacgaccaacaatccaacgctgcaaaccacgccaaccgatgaccagttcaccaataatggcggtcgtgtcgatgcggtgtacattgtggcaacgccgggtgaaatcgcttttatcaaaccgatgatcgccatgcgtaacggtagccagagcggtgcaacgctgtacgccagctcccgcagtgcgcaagggaccgctggcccggatttccgactggagatggaaggcttgcagtacagcgaaatcccgatgctggcaggcggtaatctaccgttaatgcagcaggcactcagcgcggtgaataacgattattcactggctcgcatgtatgcgatgggcgtcgatgcctggtcgctggcaaatcatttctcacaaatgcgccaggttcagggttttgaaatcaacggtaataccggaagcctgacggctaacccggattgcgtgattaacaggaacttatcatggctacagtaccaacaaggtcaggtagtccccgtcagttaa

SEQ ID NO: 81 - DNA, 78 bp, Escherichia coli
atggtaccctcaacattttctcgtttgaaagccgcgcgttgtctgcctgttgttctggcagccctgattttcgccggt

SEQ ID NO: 82 - DNA, 585 bp, Escherichia coli
tgtgtggggcaacgtgaacctgcaccggtagaagaagtgaaaccagcgccggaacaaccagccgagccacaacagcctgtccccacagtgccctcggtgccgacgatcccgcagcagccaggcccaattgagcacgaagatcaaactgcaccgcctgcgccgcatattcgccattatgactggaatggcgcaatgcagccgatggtcagtaagatgcttggggctgacggggtgactgcgggtagcgtcctgctggttgatagcgttaacaaccgtactaacggttcgctgaatgccgcagaagcgaccgaaacgctgcgaaatgcgctggctaataacgggaaatttaccctggtttccgcccagcaactgtcgatggcgaagcaacagttaggtttgtcgccgcaggacagtttaggcacccgtagtaaagccataggcattgcccgcaatgtcggcgctcattacgtgctgtactccagcgcctctggcaacgttaacgctccgaccctacaaatgcagctgatgctggtgcagacgggcgaaattatctggtcaggtaaaggtgccgtttcgcagcaataa

SEQ ID NO: 83 - DNA, 57 bp, Escherichia coli
atgacaaaaatgagtcgctacgccttgattaccgcgctggcgatgtttctcgccggg